European Patent Application EP 4 242 233 A1, published September 13, 2023. Title: ANTIBODIES FOR BINDING TO Fc ALPHA RECEPTOR. Applicant: Korea University Research and Business Foundation. The sequence listing filed with the application follows.

SEQUENCE LISTING (72 sequences)

SEQ ID NO: 1 - protein, 8 aa, Artificial Sequence
  CDRH1-JS40-1, JS48-1, JS116, JS144, JS140, JS19, JS40, JS48
GFTFSNFA

SEQ ID NO: 2 - protein, 8 aa, Artificial Sequence
  CDRH1-JS9
GFNFDDHA

SEQ ID NO: 3 - protein, 9 aa, Artificial Sequence
  CDRH1-JS30, JS41
GGSISSRDW

SEQ ID NO: 4 - protein, 8 aa, Artificial Sequence
  CDRH2-JS40-1, JS48-1, JS116, JS144, JS19, JS40, JS48
ISDDGTIT

SEQ ID NO: 5 - protein, 8 aa, Artificial Sequence
  CDRH2-JS140
ISDDGTTT

SEQ ID NO: 6 - protein, 8 aa, Artificial Sequence
  CDRH2-JS9
ISGSGGDT

SEQ ID NO: 7 - protein, 7 aa, Artificial Sequence
  CDRH2-JS30, JS41
IYHSGTT

SEQ ID NO: 8 - protein, 14 aa, Artificial Sequence
  CDRH3-JS116
VRVPPPAPVQGPDY

SEQ ID NO: 9 - protein, 14 aa, Artificial Sequence
  CDRH3-JS144
VRVPSPAPVQGPDY

SEQ ID NO: 10 - protein, 14 aa, Artificial Sequence
  CDRH3-JS140
VRVPSPAPMQGPDY

SEQ ID NO: 11 - protein, 14 aa, Artificial Sequence
  CDRH3-JS40-1, JS48-1, JS40, JS48
VKVPSPAPMQGPDY

SEQ ID NO: 12 - protein, 9 aa, Artificial Sequence
  CDRH3-JS9
ATEARGLAH

SEQ ID NO: 13 - protein, 12 aa, Artificial Sequence
  CDRH3-JS30
VTYSASDAAFDS

SEQ ID NO: 14 - protein, 12 aa, Artificial Sequence
  CDRH3-JS41
VTYSAYDAAFDS

SEQ ID NO: 15 - protein, 14 aa, Artificial Sequence
  CDRH3-JS19
VKVPSPAPMQGPDH

SEQ ID NO: 16 - protein, 10 aa, Artificial Sequence
  CDRL1-JS116, JS144, JS40-1, JS40
QGISNYLAWF

SEQ ID NO: 17 - protein, 10 aa, Artificial Sequence
  CDRL1-JS140, JS48-1, JS48
QSISTYLNWY

SEQ ID NO: 18 - protein, 10 aa, Artificial Sequence
  CDRL1-JS9
KLGERYACWY

SEQ ID NO: 19 - protein, 10 aa, Artificial Sequence
  CDRL1-JS30
QSISTCLNWY

SEQ ID NO: 20 - protein, 10 aa, Artificial Sequence
  CDRL1-JS41
QSISTYLSWY

SEQ ID NO: 21 - protein, 12 aa, Artificial Sequence
  CDRL1-JS19
SSNIGSNTVNRY

SEQ ID NO: 22 - protein, 10 aa, Artificial Sequence
  CDRL2-JS116, JS144
AASSLQGGVP

SEQ ID NO: 23 - protein, 10 aa, Artificial Sequence
  CDRL2-JS140, JS48-1, JS41, JS48
GASNLQSGVS

SEQ ID NO: 24 - protein, 10 aa, Artificial Sequence
  CDRL2-JS40-1, JS40
AASSLQSGVP

SEQ ID NO: 25 - protein, 9 aa, Artificial Sequence
  CDRL2-JS9
QDTKRPSGI

SEQ ID NO: 26 - protein, 10 aa, Artificial Sequence
  CDRL2-JS30
GASILQSGVS

SEQ ID NO: 27 - protein, 10 aa, Artificial Sequence
  CDRL2-JS19
SDNQRPSGVP

SEQ ID NO: 28 - protein, 9 aa, Artificial Sequence
  CDRL3-JS116, JS144, JS40-1, JS40
QQYHSYPLT

SEQ ID NO: 29 - protein, 9 aa, Artificial Sequence
  CDRL3-JS140
QQGNNVPLT

SEQ ID NO: 30 - protein, 9 aa, Artificial Sequence
  CDRL3-JS48-1, JS30, JS41, JS48
QQGNSVPLT

SEQ ID NO: 31 - protein, 9 aa, Artificial Sequence
  CDRL3-JS9
QAWDSSTVV

SEQ ID NO: 32 - protein, 13 aa, Artificial Sequence
  CDRL3-JS19
AVWDDSLNGPGYV

SEQ ID NO: 33 - protein, 25 aa, Artificial Sequence
  VH-FR1-JS116, JS144, JS48-1, JS40, JS19
QVQLQESGGGLVQPGGSLRLACAGS

SEQ ID NO: 34 - protein, 25 aa, Artificial Sequence
  VH-FR1-JS140, JS40-1, JS48
QVQLQESGGGLVQPGGSLRLTCAGS

SEQ ID NO: 35 - protein, 25 aa, Artificial Sequence
  VH-FR1-JS9
EVQLVGSGGGVVQPGRSLRLSCAAS

SEQ ID NO: 36 - protein, 25 aa, Artificial Sequence
  VH-FR1-JS30, JS41
EVQLVESGPGQVKPSETLSLTCSVS

SEQ ID NO: 37 - protein, 17 aa, Artificial Sequence
  VH-FR2-JS116, JS144, JS40-1, JS48-1, JS40, JS48
MAWVRLAPGKGLEWVSG

SEQ ID NO: 38 - protein, 17 aa, Artificial Sequence
  VH-FR2-JS140
MAWVRLAPGEGLEWVSG

SEQ ID NO: 39 - protein, 17 aa, Artificial Sequence
  VH-FR2-JS9
MHWVRQAPGKGLEWVSS

SEQ ID NO: 40 - protein, 17 aa, Artificial Sequence
  VH-FR2-JS30, JS41
WGWVRQPPGEGLEWIGE

SEQ ID NO: 41 - protein, 17 aa, Artificial Sequence
  VH-FR2-JS19
MAWVRQAPGKGLEWVSG

SEQ ID NO: 42 - protein, 38 aa, Artificial Sequence
  VH-FR3-JS116, JS144, JS140, JS40-1, JS48-1, JS19, JS40, JS48
DYADSVKGRFTISRDNSKNTLYLQMNSLRAEDTAVYYC

SEQ ID NO: 43 - protein, 38 aa, Artificial Sequence
  VH-FR3-JS9
YYADSVKGRFTIARDNSKNTLYLQMNSLRAEDTAVYYC

SEQ ID NO: 44 - protein, 38 aa, Artificial Sequence
  VH-FR3-JS30, JS41
NYNPSLKSRVTMSMDTSKNQLSLKLTGVTAVDTAVYYC

SEQ ID NO: 45 - protein, 11 aa, Artificial Sequence
  VH-FR4-JS116, JS144, JS48-1
WGQGTTVTVSS

SEQ ID NO: 46 - protein, 11 aa, Artificial Sequence
  VH-FR4-JS140, JS40-1, JS9, JS30, JS41, JS19, JS40, JS48
WGQGTLVTVSS

SEQ ID NO: 47 - protein, 26 aa, Artificial Sequence
  VL-FR1-JS116, JS144, JS48-1, JS40
DVVMTQSPSAMSASVGDRVTITCRAS

SEQ ID NO: 48 - protein, 26 aa, Artificial Sequence
  VL-FR1-JS140
ETTLTQSPSSLSASVGDRVSITCRAS

SEQ ID NO: 49 - protein, 26 aa, Artificial Sequence
  VL-FR1-JS40-1, JS48
ETTLTQSPSSLSASVGDRVTITCRAS

SEQ ID NO: 50 - protein, 25 aa, Artificial Sequence
  VL-FR1-JS9
SSELTQDPAVSVALGQTASITCSGH

SEQ ID NO: 51 - protein, 26 aa, Artificial Sequence
  VL-FR1-JS30, JS41
ETTLTQSPSSLSASVGDRITITCRAS

SEQ ID NO: 52 - protein, 25 aa, Artificial Sequence
  VL-FR1-JS19
QSALTQPPSASGTPGQRVTISCSGS

SEQ ID NO: 53 - protein, 13 aa, Artificial Sequence
  VL-FR2-JS116, JS144, JS48-1, JS40
QQKPGKVPKRLIY

SEQ ID NO: 54 - protein, 13 aa, Artificial Sequence
  VL-FR2-JS140, JS40-1, JS30, JS41, JS48
QQKPGKAPKSLIY

SEQ ID NO: 55 - protein, 13 aa, Artificial Sequence
  VL-FR2-JS9
QQKPGQSPVLVIY

SEQ ID NO: 56 - protein, 13 aa, Artificial Sequence
  VL-FR2-JS19
QQLPGTAPKLLIY

SEQ ID NO: 57 - protein, 29 aa, Artificial Sequence
  VL-FR3-JS116, JS144, JS48-1, JS40
SRFRGRGSGTDFTLSISCLQSEDFATYYC

SEQ ID NO: 58 - protein, 29 aa, Artificial Sequence
  VL-FR3-JS140
SQFSGRGPGADFTLTISSLQPEDFATYYC

SEQ ID NO: 59 - protein, 29 aa, Artificial Sequence
  VL-FR3-JS40-1, JS48
SQFSGRGPGTDFTLTISSLQPEDFATYYC

SEQ ID NO: 60 - protein, 30 aa, Artificial Sequence
  VL-FR3-JS9
PERFSGSNTGNTATLTITGTQAMDEADYYC

SEQ ID NO: 61 - protein, 29 aa, Artificial Sequence
  VL-FR3-JS30
SQFSGSGPGTDFTLTIGSLQPEGFATYYC

SEQ ID NO: 62 - protein, 29 aa, Artificial Sequence
  VL-FR3-JS41
SQFRGSGPGTDFTLTISSLQPEDFATYYC

SEQ ID NO: 63 - protein, 29 aa, Artificial Sequence
  VL-FR3-JS19
DRFSGSKSGTSASLAISGLQSEDEADYYC

SEQ ID NO: 64 - protein, 11 aa, Artificial Sequence
  VL-FR4-JS116, JS144, JS48-1, JS40
FGGGTKLSVLG

SEQ ID NO: 65 - protein, 11 aa, Artificial Sequence
  VL-FR4-JS140, JS40-1, JS30, JS41, JS48
FGGGTKVDIKR

SEQ ID NO: 66 - protein, 11 aa, Artificial Sequence
  VL-FR4-JS9
FGGGTKLTVLG

SEQ ID NO: 67 - protein, 11 aa, Artificial Sequence
  VL-FR4-JS19
FGTGTKVEIKR

SEQ ID NO: 68 - protein, 106 aa, Artificial Sequence
  CL
TVAAPSVFIFPPSDEQLKSGTASVVCLLNNFYPREAKVQWKVDNALQSGNSQESVTEQDSKDSTYSLSSTLTLSKADYEKHKVYACEVTHQGLSSPVTKSFNRGEC

SEQ ID NO: 69 - protein, 98 aa, Artificial Sequence
  CH1
ASTKGPSVFPLAPSSKSTSGGTAALGCLVKDYFPEPVTVSWNSGALTSGVHTFPAVLQSSGLYSLSSVVTVPSSSLGTQTYICNVNHKPSNTKVDKKV

SEQ ID NO: 70 - protein, 126 aa, Artificial Sequence
  CH2
EPPKSCDKTHTCPPCPAPELLGGPSVFLFPPKPKDTLMISRTPEVTCVVVDVSHEDPEVKFNWYVDGVEVHNAKTKPREEQYNSTYRVVSVLTVLHQDWLNGKEYKCKVSNKALPAPIEKTISKAK

SEQ ID NO: 71 - protein, 107 aa, Artificial Sequence
  CH3
GQPREPQVYTLPPSRDELTKNQVSLTCLVKGFYPSDIAVEWESNGQPENNYKTTPPVLDSDGSFFLYSKLTVDKSRWQQGNVFSCSVMHEALHNHYTQKSLSLSPGK

SEQ ID NO: 72 - protein, 206 aa, Homo sapiens
QEGDFPMPFISAKSSPVIPLDGSVKIQCQAIREAYLTQLMIIKNSTYREIGRRLKFWNETDPEFVIDHMDANKAGRYQCQYRIGHYRFRYSDTLELVVTGLYGKPFLSADRGLVLMPGENISLTCSSAHIPFDRFSLAKEGELSLPQHQSGEHPANFSLGPVDLNVSGIYRCYGWYNRSPYLWSFPSNALELVVTDSIHQDYTTQN